European Patent Application EP 4 357 361 A1, published April 24, 2024. Title: 抗IL-36R的抗体及其用途. Applicant: 正大天晴药业集团股份有限公司. The sequence listing filed with the application follows.

SEQUENCE LISTING (90 sequences)

SEQ ID NO: 1 - protein, 10 aa, 人工序列(Artificial Sequence)
  小鼠、嵌合和人源化72C1抗体的VH-CDR1
GASITSGYWN

SEQ ID NO: 2 - protein, 16 aa, 人工序列(Artificial Sequence)
  UNSURE (3): Xaa = S or Y
  小鼠、嵌合和人源化72C1抗体的VH-CDR2
YIXYSGYTYYNPSLKS

SEQ ID NO: 3 - protein, 12 aa, 人工序列(Artificial Sequence)
  小鼠、嵌合和人源化72C1抗体的VH-CDR3
GGYDYVEDALYY

SEQ ID NO: 4 - protein, 10 aa, 人工序列(Artificial Sequence)
  小鼠、嵌合和人源化72C1抗体的VL-CDR1
RASSNVRYMY

SEQ ID NO: 5 - protein, 7 aa, 人工序列(Artificial Sequence)
  小鼠、嵌合和人源化72C1抗体的VL-CDR2
LTSNLAS

SEQ ID NO: 6 - protein, 9 aa, 人工序列(Artificial Sequence)
  UNSURE (3): Xaa = F or Y
  小鼠、嵌合和人源化72C1抗体的VL-CDR3
QQXTTSPYT

SEQ ID NO: 7 - protein, 120 aa, 人工序列(Artificial Sequence)
  小鼠和嵌合72C1抗体的VH
EVQLQQSGPSLVKPSQTLSLTCSVTGASITSGYWNWIRNFPGNKLEYMGYISYSGYTYYNPSLKSRISITRDTSKNQYYLQLISVTTEDTATYYCATGGYDYVEDALYYWGQGTSVTVSS

SEQ ID NO: 8 - DNA, 360 bp, 人工序列(Artificial Sequence)
  嵌合72C1抗体的VH
gaggtgcagctgcagcagtccggcccctctctggtgaagccttctcagaccctgagcctgacatgctccgtgaccggcgccagcatcacatccggctactggaactggatccggaatttcccaggcaacaagctggagtacatgggctatatctcttacagcggctatacctactataatccctctctgaagagccggatctccatcaccagagacacatctaagaaccagtactatctgcagctgatctccgtgaccacagaggataccgccacatactattgtgccacaggcggctacgactatgtggaggatgccctgtactattggggccagggcaccagcgtgacagtgagctcc

SEQ ID NO: 9 - protein, 120 aa, 人工序列(Artificial Sequence)
  hz72C1-1.1和hz72C1-2.1抗体的VH
QVQLQESGPGLVKPSQTLSLTCTVSGASITSGYWNWIRNHPGKGLEYIGYISYSGYTYYNPSLKSRVTISRDTSKNQFSLKLSSVTAADTAVYYCATGGYDYVEDALYYWGQGTLVTVSS

SEQ ID NO: 10 - DNA, 360 bp, 人工序列(Artificial Sequence)
  hz72C1-1.1和hz72C1-2.1抗体的VH
caggtgcagctgcaggagtccggaccaggactggtgaagccttctcagaccctgtccctgacctgcacagtgtccggcgccagcatcacatctggctactggaactggatcaggaatcacccaggcaagggcctggagtacatcggctatatcagctactctggctatacctactataacccctccctgaagagcagggtgaccatcagccgggacacatctaagaatcagttctccctgaagctgtccagcgtgaccgccgctgatacagccgtgtactattgtgctacaggcggctacgactatgtggaggatgctctgtactattggggccagggcaccctggtgacagtgtcttcc

SEQ ID NO: 11 - protein, 120 aa, 人工序列(Artificial Sequence)
  hz72C1-1.2和hz72C1-2.2抗体的VH
QVQLQESGPGLVKPSQTLSLTCTVSGASITSGYWNWIRNHPGKGLEYIGYISYSGYTYYNPSLKSRVTISRDTSKNQYYLKLSSVTAADTAVYYCATGGYDYVEDALYYWGQGTLVTVSS

SEQ ID NO: 12 - DNA, 360 bp, 人工序列(Artificial Sequence)
  hz72C1-1.2和hz72C1-2.2抗体的VH
caggtgcagctgcaggagtccggaccaggactggtgaagccttctcagaccctgtccctgacctgcacagtgtccggcgccagcatcacatctggctactggaactggatcaggaatcacccaggcaagggcctggagtacatcggctatatcagctactctggctatacctactataacccctccctgaagagcagggtgaccatcagccgggacacatctaagaatcagtactatctgaagctgtccagcgtgaccgccgctgatacagccgtgtactattgtgctacaggcggctacgactatgtggaggatgctctgtactattggggccagggcaccctggtgacagtgtcttcc

SEQ ID NO: 13 - protein, 120 aa, 人工序列(Artificial Sequence)
  hz72C1-1.3和hz72C1-2.3抗体的VH
QVQLQESGPGLVKPSQTLSLTCTVSGASITSGYWNWIRNHPGKGLEYIGYIYYSGYTYYNPSLKSRVTISRDTSKNQYYLKLSSVTAADTAVYYCATGGYDYVEDALYYWGQGTLVTVSS

SEQ ID NO: 14 - DNA, 360 bp, 人工序列(Artificial Sequence)
  hz72C1-1.3和hz72C1-2.3抗体的VH
caggtgcagctgcaggagagcggaccaggactggtgaagccttcccagaccctgagcctgacctgcacagtgagcggcgcctctatcacatccggctactggaactggatcaggaatcacccaggcaagggcctggagtacatcggctatatctactattctggctatacctactataaccccagcctgaagtctagggtgaccatctctcgggacacatccaagaatcagtactatctgaagctgtccagcgtgaccgccgctgatacagccgtgtactattgtgctacaggcggctacgactatgtggaggatgctctgtactattggggccagggcaccctggtgacagtgtcttcc

SEQ ID NO: 15 - protein, 106 aa, 人工序列(Artificial Sequence)
  小鼠和嵌合72C1抗体的VL
EILLTQSPAIMSATLGEKVTMSCRASSNVRYMYWYQLKSGASPKLWIYLTSNLASGVPARFSGSGSGTSYSLTISSVEAEDAATYFCQQFTTSPYTFGGGTKLEIK

SEQ ID NO: 16 - DNA, 318 bp, 人工序列(Artificial Sequence)
  嵌合72C1抗体的VL
gagatcctgctgacccagtccccagccatcatgtctgccaccctgggcgagaaggtgacaatgtcctgccgggccagctccaacgtgagatacatgtattggtaccagctgaagagcggcgcctcccccaagctgtggatctatctgacctctaatctggcaagcggagtgcctgcacggttctccggctctggcagcggcacctcctactctctgacaatctctagcgtggaggcagaggacgcagcaacatatttctgtcagcagtttaccacaagcccctacacctttggcggcggcacaaagctggagatcaag

SEQ ID NO: 17 - protein, 106 aa, 人工序列(Artificial Sequence)
  hz72C1-1.1、hz72C1-1.2和hz72C1-1.3抗体的VL
DIQMTQSPSSLSASVGDRVTITCRASSNVRYMYWYQQKPGKAPKLWIYLTSNLASGVPSRFSGSGSGTSYTLTISSLQPEDFATYYCQQFTTSPYTFGQGTKLEIK

SEQ ID NO: 18 - DNA, 318 bp, 人工序列(Artificial Sequence)
  hz72C1-1.1、hz72C1-1.2和hz72C1-1.3抗体的VL
gacatccagatgacccagtccccttccagcctgtccgccagcgtgggcgatagggtgaccatcacatgccgggcttcttccaacgtgagatacatgtattggtaccagcagaagcccggcaaggcccctaagctgtggatctatctgacatctaatctggcttccggagtgccaagccgcttctctggatccggaagcggcacctcttacaccctgacaatcagctctctgcagccagaggactttgccacatactattgtcagcagttcaccacatccccctatacctttggccagggcacaaagctggagatcaag

SEQ ID NO: 19 - protein, 106 aa, 人工序列(Artificial Sequence)
  hz72C1-2.1、hz72C1-2.2和hz72C1-2.3抗体的VL
DIQMTQSPSSLSASVGDRVTITCRASSNVRYMYWYQQKPGKAPKLWIYLTSNLASGVPSRFSGSGSGTSYTLTISSLQPEDFATYYCQQYTTSPYTFGQGTKLEIK

SEQ ID NO: 20 - DNA, 318 bp, 人工序列(Artificial Sequence)
  hz72C1-2.1、hz72C1-2.2和hz72C1-2.3抗体的VL
gacatccagatgacccagtccccttccagcctgtccgccagcgtgggcgatagggtgaccatcacatgccgggcttcttccaacgtgagatacatgtattggtaccagcagaagcccggcaaggcccctaagctgtggatctatctgacatctaatctggcttccggagtgccaagccgcttctctggatccggaagcggcacctcttacaccctgacaatcagctctctgcagccagaggacttcgccacatactattgtcagcagtataccacatccccctacacctttggccagggcacaaagctggagatcaag

SEQ ID NO: 21 - protein, 10 aa, 人工序列(Artificial Sequence)
  UNSURE (3): Xaa = F or Y
  小鼠、嵌合和人源化84C4抗体的VH-CDR1
GYXFTSYWMN

SEQ ID NO: 22 - protein, 17 aa, 人工序列(Artificial Sequence)
  UNSURE (1): Xaa = M or Y
  UNSURE (3): Xaa = H or Y
  UNSURE (11): Xaa = L or Y
  UNSURE (12): Xaa = N or A
  UNSURE (16): Xaa = K or Q
  小鼠、嵌合和人源化84C4抗体的VH-CDR2
XIXPYDSETRXXQKFXG

SEQ ID NO: 23 - protein, 7 aa, 人工序列(Artificial Sequence)
  小鼠、嵌合和人源化84C4抗体的VH-CDR3
STTAFAY

SEQ ID NO: 24 - protein, 10 aa, 人工序列(Artificial Sequence)
  小鼠、嵌合和人源化84C4抗体的VL-CDR1
ASQDIGNALN

SEQ ID NO: 25 - protein, 7 aa, 人工序列(Artificial Sequence)
  小鼠、嵌合和人源化84C4抗体的VL-CDR2
ATSSLDP

SEQ ID NO: 26 - protein, 9 aa, 人工序列(Artificial Sequence)
  小鼠、嵌合和人源化84C4抗体的VL-CDR3
LQYASSPYT

SEQ ID NO: 27 - protein, 116 aa, 人工序列(Artificial Sequence)
  小鼠和嵌合84C4抗体的VH
EVQLQQLGAELVRPGASVMLSCKVSGYFFTSYWMNWVNQRPGQGLEWIGMIHPYDSETRLNQKFKGKATLTVDKSASTAYLQLSSPTSEEYAVYYCASSTTAFAYWGQGTLVTVSA

SEQ ID NO: 28 - DNA, 348 bp, 人工序列(Artificial Sequence)
  嵌合84C4抗体的VH
gaggtgcagctgcagcagctgggagcagagctggtgcggccaggagcaagcgtgatgctgtcctgcaaggtgtctggctacttctttaccagctattggatgaactgggtgaatcagaggccaggacagggactggagtggatcggcatgatccacccttacgactccgagacaagactgaaccagaagttcaagggcaaggccaccctgacagtggataagtccgcctctaccgcctacctgcagctgagctcccccacatctgaggagtatgccgtgtactattgtgcctctagcaccacagcctttgcctattggggccagggcaccctggtgacagtgagcgcc

SEQ ID NO: 29 - protein, 116 aa, 人工序列(Artificial Sequence)
  hz84C4-1.1和hz84C4-2.1抗体的VH
QVQLVQSGAEVKKPGASVKVSCKASGYFFTSYWMNWVRQAPGQGLEWMGMIHPYDSETRYAQKFQGRVTMTVDKSTSTVYMELSSLRSEDTAVYYCASSTTAFAYWGQGTLVTVSS

SEQ ID NO: 30 - DNA, 348 bp, 人工序列(Artificial Sequence)
  hz84C4-1.1和hz84C4-2.1抗体的VH
caagtgcagctggtgcagagcggagccgaggtgaaaaagcccggcgcttctgtgaaggtgtcctgcaaggccagcggctacttcttcacctcctactggatgaactgggtgcggcaggcccctggccagggcctggaatggatgggcatgatccacccttacgacagcgagacaagatacgcccagaagttccagggcagagtgaccatgaccgtggataagagcaccagcacagtgtatatggaactgagcagcctgagaagcgaggacaccgccgtgtactactgtgcctcttctacaaccgcttttgcctactggggccagggaaccctggttacagtcagcagc

SEQ ID NO: 31 - protein, 116 aa, 人工序列(Artificial Sequence)
  hz84C4-1.2和hz84C4-2.2抗体的VH
QVQLVQSGAEVKKPGASVKVSCKASGYFFTSYWMNWVRQAPGQGLEWMGYIHPYDSETRYAQKFQGRVTMTVDKSTSTVYMELSSLRSEDTAVYYCASSTTAFAYWGQGTLVTVSS

SEQ ID NO: 32 - DNA, 348 bp, 人工序列(Artificial Sequence)
  hz84C4-1.2和hz84C4-2.2抗体的VH
caagtgcagctggttcagagcggcgccgaggtgaagaagcctggcgctagcgtgaaggtgtcttgtaaagcctctggctacttcttcaccagctactggatgaactgggtcagacaggcccctggccagggcctggaatggatgggatatatccacccctacgacagcgagacaagatacgcccagaagttccagggcagagtgacaatgaccgtggacaagtccacctctacagtgtacatggaactgagcagcctgcggagcgaggataccgccgtgtactactgcgccagcagcaccaccgcttttgcctactggggccagggaacactggtgaccgtgtccagc

SEQ ID NO: 33 - protein, 116 aa, 人工序列(Artificial Sequence)
  hz84C4-1.3和hz84C4-2.3抗体的VH
QVQLVQSGAEVKKPGASVKVSCKASGYFFTSYWMNWVRQAPGQGLEWMGMIYPYDSETRYAQKFQGRVTMTVDKSTSTVYMELSSLRSEDTAVYYCASSTTAFAYWGQGTLVTVSS

SEQ ID NO: 34 - DNA, 348 bp, 人工序列(Artificial Sequence)
  hz84C4-1.3和hz84C4-2.3抗体的VH
caagtgcagctggttcagagcggcgccgaggtgaaaaagcctggcgcttctgtgaaggtgtcctgcaaggcctctggctacttcttcacctcctactggatgaactgggtgcggcaggcccctggacagggcctggaatggatgggcatgatctacccctacgacagcgagacaagatacgcccagaagttccagggaagagtgacaatgaccgtggataagagcaccagcacagtgtatatggaactgagcagcctgagaagcgaggacaccgccgtgtactactgtgccagcagcaccacagcttttgcctactggggccagggcaccctggtgaccgtcagctct

SEQ ID NO: 35 - protein, 116 aa, 人工序列(Artificial Sequence)
  hz84C4-1.4和hz84C4-2.4抗体的VH
QVQLVQSGAEVKKPGASVKVSCKASGYYFTSYWMNWVRQAPGQGLEWMGMIHPYDSETRLAQKFKGRVTMTVDKSTSTVYMELSSLRSEDTAVYYCASSTTAFAYWGQGTLVTVSS

SEQ ID NO: 36 - DNA, 348 bp, 人工序列(Artificial Sequence)
  hz84C4-1.4和hz84C4-2.4抗体的VH
caagtgcagctggtccagagcggcgccgaggtgaaaaagcctggagcttctgtgaaggtgtcctgcaaggcctccggctactacttcaccagctactggatgaactgggtgcggcaggcccctggccagggcctggaatggatgggcatgatccacccctacgacagcgagacaagactggcccagaaattcaagggcagagtgaccatgaccgtggataagagcacaagcaccgtgtacatggaactgagcagcctgagaagcgaggacaccgccgtgtactattgtgcctctagcaccaccgcttttgcctactggggccagggaacactggtgacagtttctagc

SEQ ID NO: 37 - protein, 116 aa, 人工序列(Artificial Sequence)
  hz84C4-1.5和hz84C4-2.5抗体的VH
QVQLVQSGAEVKKPGASVKVSCKVSGYFFTSYWMNWVNQAPGQGLEWMGMIHPYDSETRLAQKFKGRVTMTVDKSTSTVYMELSSLRSEDTAVYYCASSTTAFAYWGQGTLVTVSS

SEQ ID NO: 38 - DNA, 348 bp, 人工序列(Artificial Sequence)
  hz84C4-1.5和hz84C4-2.5抗体的VH
caagtgcagctggttcagagcggcgccgaggtgaaaaagcctggcgcttctgtgaaggtgtcttgtaaagtgtccggatatttcttcaccagctactggatgaactgggtcaaccaggcccctggacagggcctggaatggatgggcatgatccacccctacgacagcgagacaagactggcccagaagttcaagggcagagtgaccatgaccgtggataagagcacctctaccgtgtacatggaactgagcagcctgcggagcgaggacaccgccgtgtactactgcgccagcagcacaacagcttttgcctactggggccagggcaccctggtgacagtgtccagc

SEQ ID NO: 39 - protein, 107 aa, 人工序列(Artificial Sequence)
  小鼠和嵌合84C4抗体的VL
DILMTQSPSSLSASLGERVSLTCRASQDIGNALNWLQQAPDGTIKRLIYATSSLDPGVPKRFSGSRSGSDYSLTISSLASEDFVYYYCLQYASSPYTFGGGTKLEIK

SEQ ID NO: 40 - DNA, 321 bp, 人工序列(Artificial Sequence)
  嵌合84C4抗体的VL
gacatcctgatgacccagagcccaagctccctgtctgccagcctgggagagagggtgtctctgacatgcagggcaagccaggacatcggaaacgccctgaattggctgcagcaggcccccgatggcaccatcaagcggctgatctatgccacatctagcctggatcccggcgtgcctaagcggttctccggctctagaagcggctccgactactccctgaccatctcctctctggcctctgaggatttcgtgtactattactgtctgcagtatgcaagctccccatacacctttggcggaggaacaaagctggagatcaag

SEQ ID NO: 41 - protein, 107 aa, 人工序列(Artificial Sequence)
  hz84C4-1.1、hz84C4-1.2、hz84C4-1.3、hz84C4-1.4和hz84C4-1.5抗体的VL
DIQMTQSPSSLSASVGDRVTITCRASQDIGNALNWYQQKPGKAPKRLIYATSSLDPGVPSRFSGSRSGTDFTLTISSLQPEDFATYYCLQYASSPYTFGQGTKVEIK

SEQ ID NO: 42 - DNA, 321 bp, 人工序列(Artificial Sequence)
  hz84C4-1.1、hz84C4-1.2、hz84C4-1.3、hz84C4-1.4和hz84C4-1.5抗体的VL
gatattcagatgacccagagcccttcctccctgagcgctagcgtgggcgacagagtgaccatcacctgtagagcctctcaggacatcggcaacgccctgaactggtaccagcagaaacctggcaaggcccctaagcggctgatctacgccaccagcagcctggaccccggagtccccagcagattcagcggcagccggagcggaacagattttaccctgaccatcagctccctgcaacctgaggacttcgccacatactactgcctgcagtacgcttcttctccatatacattcggccagggcaccaaggtggaaatcaag

SEQ ID NO: 43 - protein, 107 aa, 人工序列(Artificial Sequence)
  hz84C4-2.1、hz84C4-2.2、hz84C4-2.3、hz84C4-2.4和hz84C4-2.5抗体的VL
DIQMTQSPSSLSASVGDRVTITCRASQDIGNALNWLQQKPGKAPKRLIYATSSLDPGVPSRFSGSRSGTDYTLTISSLQPEDFATYYCLQYASSPYTFGQGTKVEIK

SEQ ID NO: 44 - DNA, 321 bp, 人工序列(Artificial Sequence)
  hz84C4-2.1、hz84C4-2.2、hz84C4-2.3、hz84C4-2.4和hz84C4-2.5抗体的VL
gatattcagatgacccagagcccatcttccctgagcgccagcgtgggcgatagagtgaccatcacctgtagagcctcccaggacatcggcaacgccctgaactggctgcagcagaaacctggcaaggcccctaagcggctgatctacgctacaagctccctcgaccccggcgtccccagcagattcagcggatctcggagcggaacagactacaccctgaccatcagcagcctgcaacctgaggacttcgccacctactactgcctgcagtacgcttctagcccttatacctttggccagggcacaaaggtggaaatcaag

SEQ ID NO: 45 - protein, 10 aa, 人工序列(Artificial Sequence)
  小鼠和嵌合74B4D6抗体的VH-CDR1
GYTFTNYWIH

SEQ ID NO: 46 - protein, 17 aa, 人工序列(Artificial Sequence)
  小鼠和嵌合74B4D6抗体的VH-CDR2
TIDPSENYTNYNQKFKG

SEQ ID NO: 47 - protein, 5 aa, 人工序列(Artificial Sequence)
  小鼠和嵌合74B4D6抗体的VH-CDR3
SSFSY

SEQ ID NO: 48 - protein, 10 aa, 人工序列(Artificial Sequence)
  小鼠和嵌合74B4D6抗体的VL-CDR1
SASSSVSFIH

SEQ ID NO: 49 - protein, 7 aa, 人工序列(Artificial Sequence)
  小鼠和嵌合74B4D6抗体的VL-CDR2
TTSNLAS

SEQ ID NO: 50 - protein, 9 aa, 人工序列(Artificial Sequence)
  小鼠和嵌合74B4D6抗体的VL-CDR3
QQRSSYPLT

SEQ ID NO: 51 - protein, 114 aa, 人工序列(Artificial Sequence)
  小鼠和嵌合74B4D6抗体的VH
EVQLQQPGAELGKPGASVKMACKASGYTFTNYWIHWVKQRPGQGLEWIGTIDPSENYTNYNQKFKGKATLTVDTSSSTAYMQLSSLTSEDKAVYFCTGSSFSYWGQGTLVTVSA

SEQ ID NO: 52 - protein, 106 aa, 人工序列(Artificial Sequence)
  小鼠和嵌合74B4D6抗体的VL
QNVLTQSPAIMSVSPGEKVTMTCSASSSVSFIHWFQQKPGTSPKLWIYTTSNLASGVPARFSGSGSGTSYSLTISRMEAEDAATYYCQQRSSYPLTFGAGTKLELK

SEQ ID NO: 53 - protein, 10 aa, 人工序列(Artificial Sequence)
  小鼠和嵌合58A8D1抗体的VH-CDR1
GYSFTSSWMH

SEQ ID NO: 54 - protein, 17 aa, 人工序列(Artificial Sequence)
  小鼠和嵌合58A8D1抗体的VH-CDR2
EIHPNSGNTNYNEKFKG

SEQ ID NO: 55 - protein, 11 aa, 人工序列(Artificial Sequence)
  小鼠和嵌合58A8D1抗体的VH-CDR3
SPYGYGGSMDY

SEQ ID NO: 56 - protein, 11 aa, 人工序列(Artificial Sequence)
  小鼠和嵌合58A8D1抗体的VL-CDR1
RASQDIHNYLN

SEQ ID NO: 57 - protein, 7 aa, 人工序列(Artificial Sequence)
  小鼠和嵌合58A8D1抗体的VL-CDR2
YTSRLYS

SEQ ID NO: 58 - protein, 9 aa, 人工序列(Artificial Sequence)
  小鼠和嵌合58A8D1抗体的VL-CDR3
QQGNTLPVM

SEQ ID NO: 59 - protein, 120 aa, 人工序列(Artificial Sequence)
  小鼠和嵌合58A8D1抗体的VH
EVQLQQLGSVLVRPGISVKLSCKASGYSFTSSWMHWTKQRPGQGLEWIGEIHPNSGNTNYNEKFKGKATLTVDTSSRTAYVDLSSLTSEDSAVYYCARSPYGYGGSMDYWGQGTSVTVSS

SEQ ID NO: 60 - protein, 107 aa, 人工序列(Artificial Sequence)
  小鼠和嵌合58A8D1抗体的VL
DIQMTQTTSSLSASLGDRVTISCRASQDIHNYLNWYQQKPDGTVKLLIYYTSRLYSGVPSRFSGSGSGTDYSLTISNLEQEDFATYFCQQGNTLPVMFGSGTKLELK

SEQ ID NO: 61 - protein, 10 aa, 人工序列(Artificial Sequence)
  小鼠和嵌合6G10抗体的VH-CDR1
GITFSRFAMS

SEQ ID NO: 62 - protein, 17 aa, 人工序列(Artificial Sequence)
  小鼠和嵌合6G10抗体的VH-CDR2
TISSGDMYTYYPDSVKG

SEQ ID NO: 63 - protein, 9 aa, 人工序列(Artificial Sequence)
  小鼠和嵌合6G10抗体的VH-CDR3
MITTGEHAY

SEQ ID NO: 64 - protein, 11 aa, 人工序列(Artificial Sequence)
  小鼠和嵌合6G10抗体的VL-CDR1
RASQDISVWLT

SEQ ID NO: 65 - protein, 7 aa, 人工序列(Artificial Sequence)
  小鼠和嵌合6G10抗体的VL-CDR2
KASNLHT

SEQ ID NO: 66 - protein, 9 aa, 人工序列(Artificial Sequence)
  小鼠和嵌合6G10抗体的VL-CDR3
LQSQSYPWT

SEQ ID NO: 67 - protein, 118 aa, 人工序列(Artificial Sequence)
  小鼠和嵌合6G10抗体的VH
EVMLVESGGGLVKPGGSLKLSCAASGITFSRFAMSWIRQTPEKRLEWVATISSGDMYTYYPDSVKGRFTISRDNANNTLYLQMRSLRSEDTAMYYCAIMITTGEHAYWGQGTLVTVSA

SEQ ID NO: 68 - protein, 107 aa, 人工序列(Artificial Sequence)
  小鼠和嵌合6G10抗体的VL
EIKMTQSPSSLSASLGDTITITCRASQDISVWLTWYQQKPGNIPKLLIYKASNLHTGVPPRFSGSGSGTDFTFTISSLQPEDITTYYCLQSQSYPWTFGGGTKLEIK

SEQ ID NO: 69 - protein, 330 aa, 人工序列(Artificial Sequence)
  人IgG1重链恒定区
ASTKGPSVFPLAPSSKSTSGGTAALGCLVKDYFPEPVTVSWNSGALTSGVHTFPAVLQSSGLYSLSSVVTVPSSSLGTQTYICNVNHKPSNTKVDKRVEPKSCDKTHTCPPCPAPEAAGGPSVFLFPPKPKDTLMISRTPEVTCVVVDVSHEDPEVKFNWYVDGVEVHNAKTKPREEQYNSTYRVVSVLTVLHQDWLNGKEYKCKVSNKALPAPIEKTISKAKGQPREPQVYTLPPSREEMTKNQVSLTCLVKGFYPSDIAVEWESNGQPENNYKTTPPVLDSDGSFFLYSKLTVDKSRWQQGNVFSCSVMHEALHNHYTQKSLSLSPGK

SEQ ID NO: 70 - DNA, 990 bp, 人工序列(Artificial Sequence)
  人IgG1重链恒定区
gcctctaccaagggcccctccgtgttccctctggctccaagctctaagtccaccagcggaggaacagccgctctgggctgtctggtgaaggattatttcccagagcccgtgaccgtgtcctggaatagcggcgccctgacctccggagtgcatacatttcccgctgtgctgcagtccagcggcctgtacagcctgtcttccgtggtgaccgtgcctagctcttccctgggcacccagacatatatctgcaatgtgaaccacaagccttccaacacaaaggtggacaagagggtggagccaaagagctgtgataagacccatacatgccccccttgtcctgctccagaggctgctggaggaccatccgtgttcctgtttccacccaagcccaaggacaccctgatgatctctaggacccctgaggtgacatgcgtggtggtggacgtgtcccacgaggatccagaggtgaagtttaattggtacgtggatggcgtggaggtgcataacgctaagaccaagcctagggaggagcagtacaacagcacctatcgggtggtgtctgtgctgacagtgctgcaccaggactggctgaatggcaaggagtataagtgcaaggtgagcaacaaggccctgcccgctcctatcgagaagaccatctctaaggccaagggccagcccagagagcctcaggtgtacacactgcctccaagccgcgaggagatgaccaagaatcaggtgtctctgacatgtctggtgaagggcttctatccatctgacatcgctgtggagtgggagtccaacggccagcccgagaacaattacaagaccacaccccctgtgctggactctgatggctccttctttctgtattccaagctgaccgtggataagagccggtggcagcagggcaacgtgttctcctgttccgtgatgcatgaggccctgcacaaccattacacacagaagagcctgtctctgtccccaggcaag

SEQ ID NO: 71 - protein, 327 aa, 人工序列(Artificial Sequence)
  人IgG4重链恒定区
ASTKGPSVFPLAPCSRSTSESTAALGCLVKDYFPEPVTVSWNSGALTSGVHTFPAVLQSSGLYSLSSVVTVPSSSLGTKTYTCNVDHKPSNTKVDKRVESKYGPPCPPCPAPEFLGGPSVFLFPPKPKDTLMISRTPEVTCVVVDVSQEDPEVQFNWYVDGVEVHNAKTKPREEQFNSTYRVVSVLTVLHQDWLNGKEYKCKVSNKGLPSSIEKTISKAKGQPREPQVYTLPPSQEEMTKNQVSLTCLVKGFYPSDIAVEWESNGQPENNYKTTPPVLDSDGSFFLYSRLTVDKSRWQEGNVFSCSVMHEALHNHYTQKSLSLSLGK

SEQ ID NO: 72 - DNA, 981 bp, 人工序列(Artificial Sequence)
  人IgG4重链恒定区
gccagcacaaagggaccatccgtgttcccactggctccatgctcccggagcacctctgagtccacagccgctctgggctgtctggtgaaggactacttccctgagccagtgaccgtgtcctggaatagcggcgccctgaccagcggagtgcacacatttcctgctgtgctgcagagctctggcctgtactctctgtccagcgtggtgaccgtgccatcttccagcctgggcacaaagacctatacatgcaacgtggaccataagccctccaatacaaaggtggataagagagtggagagcaagtacggaccaccttgcccaccatgtccagctcctgagtttctgggaggaccatccgtgttcctgtttcctccaaagcctaaggacaccctgatgatctccaggaccccagaggtgacatgcgtggtggtggacgtgagccaggaggatcctgaggtgcagttcaactggtacgtggatggcgtggaggtgcacaatgctaagaccaagcctagagaggagcagtttaactccacctaccgcgtggtgagcgtgctgacagtgctgcatcaggattggctgaacggcaaggagtataagtgcaaggtgtctaataagggcctgccatcttccatcgagaagaccatctccaaggccaagggccagcctagggagccacaggtgtacacactgcccccttctcaggaggagatgaccaagaaccaggtgtccctgacatgtctggtgaagggcttctatcctagcgacatcgctgtggagtgggagtctaatggccagccagagaacaattacaagaccacaccacccgtgctggactctgatggctccttctttctgtattctaggctgaccgtggataagtcccggtggcaggagggcaacgtgtttagctgctctgtgatgcatgaggctctgcacaatcattacacacagaagtccctgagcctgtctctgggcaag

SEQ ID NO: 73 - protein, 107 aa, 人工序列(Artificial Sequence) [sequence omitted]

SEQ ID NO: 74 - DNA, 321 bp, 人工序列(Artificial Sequence)
  人κ轻链恒定区
cgcacagtggccgctccaagcgtgttcatctttcccccttctgacgagcagctgaagtctggcaccgcttccgtggtgtgcctgctgaacaatttctacccccgcgaggccaaggtgcagtggaaggtggataacgctctgcagtccggcaatagccaggagtctgtgacagagcaggactccaaggatagcacctattctctgtccagcacactgaccctgtctaaggccgattacgagaagcacaaggtgtatgcttgcgaggtgacacatcagggcctgtcttccccagtgaccaagtcctttaacaggggcgagtgt

SEQ ID NO: 75 - protein, 575 aa, 人(Homo sapiens)
MWSLLLCGLSIALPLSVTADGCKDIFMKNEILSASQPFAFNCTFPPITSGEVSVTWYKNSSKIPVSKIIQSRIHQDETWILFLPMEWGDSGVYQCVIKGRDSCHRIHVNLTVFEKHWCDTSIGGLPNLSDEYKQILHLGKDDSLTCHLHFPKSCVLGPIKWYKDCNEIKGERFTVLETRLLVSNVSAEDRGNYACQAILTHSGKQYEVLNGITVSITERAGYGGSVPKIIYPKNHSIEVQLGTTLIVDCNVTDTKDNTNLRCWRVNNTLVDDYYDESKRIREGVETHVSFREHNLYTVNITFLEVKMEDYGLPFMCHAGVSTAYIILQLPAPDFRAYLIGGLIALVAVAVSVVYIYNIFKIDIVLWYRSAFHSTETIVDGKLYDAYVLYPKPHKESQRHAVDALVLNILPEVLERQCGYKLFIFGRDEFPGQAVANVIDENVKLCRRLIVIVVPESLGFGLLKNLSEEQIAVYSALIQDGMKVILIELEKIEDYTVMPESIQYIKQKHGAIRWHGDFTEQSQCMKTKFWKTVRYHMPPRRCRPFPPVQLLQHTPCYRTAGPELGSRRKKCTLTTG

SEQ ID NO: 76 - protein, 555 aa, 人工序列(Artificial Sequence)
  hIL36R-ECD mFc
DGCKDIFMKNEILSASQPFAFNCTFPPITSGEVSVTWYKNSSKIPVSKIIQSRIHQDETWILFLPMEWGDSGVYQCVIKGRDSCHRIHVNLTVFEKHWCDTSIGGLPNLSDEYKQILHLGKDDSLTCHLHFPKSCVLGPIKWYKDCNEIKGERFTVLETRLLVSNVSAEDRGNYACQAILTHSGKQYEVLNGITVSITERAGYGGSVPKIIYPKNHSIEVQLGTTLIVDCNVTDTKDNTNLRCWRVNNTLVDDYYDESKRIREGVETHVSFREHNLYTVNITFLEVKMEDYGLPFMCHAGVSTAYIILQLPAPDFRIEGRMDEPRGPTIKPCPPCKCPAPNLLGGPSVFIFPPKIKDVLMISLSPIVTCVVVDVSEDDPDVQISWFVNNVEVHTAQTQTHREDYNSTLRVVSALPIQHQDWMSGKEFKCKVNNKDLPAPIERTISKPKGSVRAPQVYVLPPPEEEMTKKQVTLTCMVTDFMPEDIYVEWTNNGKTELNYKNTEPVLDSDGSYFMYSKLRVEKKNWVERNSYSCSVVHEGLHNHHTTKSFSRTPGK

SEQ ID NO: 77 - protein, 553 aa, 人工序列(Artificial Sequence)
  hIL36R-ECD hFc
DGCKDIFMKNEILSASQPFAFNCTFPPITSGEVSVTWYKNSSKIPVSKIIQSRIHQDETWILFLPMEWGDSGVYQCVIKGRDSCHRIHVNLTVFEKHWCDTSIGGLPNLSDEYKQILHLGKDDSLTCHLHFPKSCVLGPIKWYKDCNEIKGERFTVLETRLLVSNVSAEDRGNYACQAILTHSGKQYEVLNGITVSITERAGYGGSVPKIIYPKNHSIEVQLGTTLIVDCNVTDTKDNTNLRCWRVNNTLVDDYYDESKRIREGVETHVSFREHNLYTVNITFLEVKMEDYGLPFMCHAGVSTAYIILQLPAPDFRIEGRMDPKSCDKTHTCPPCPAPELLGGPSVFLFPPKPKDTLMISRTPEVTCVVVDVSHEDPEVKFNWYVDGVEVHNAKTKPREEQYNSTYRVVSVLTVLHQDWLNGKEYKCKVSNKALPAPIEKTISKAKGQPREPQVYTLPPSRDELTKNQVSLTCLVKGFYPSDIAVEWESNGQPENNYKTTPPVLDSDGSFFLYSKLTVDKSRWQQGNVFSCSVMHEALHNHYTQKSLSLSPGK

SEQ ID NO: 78 - protein, 595 aa, 食蟹猴(Macaca fascicularis)
MWSLLLCGLSIALPLSVTADGCNDIFMKNEMLSASQPFAFNCTFPPITSGEVSVTWYKNSSKIPVSKIIQSRIHQDETWILFLPMEWGDSGVYQCVIKGRDSCHRIHVNLTVFEKQWCDTSVKGLPNLSDEYKQILHLGKDDSLTCHLHFPKSCILGPIKWYKDCNEITGERFTVLETRLLVSNVSAEDRGNYACQVILTHSGKQYEVLNGITVSITERAGYGGSVPKIIYPKNNSIEVQLGTTLIVDCNITDTKDNTNLRCWRVNNTLVDDYYNESKRIREGVETHASFREYNLYTVNITFLEVKMEDYGLPFMCHAGVSAAYIMLQLPAPDFRAYLIGGLIAFLAVAVSVVYIYNIFKIDIVLWYRSTFQSTETLEDGKLYDAYVLYPKPRRESQRHAVDTLVLKILPEVLERQCGYKLFIFGRDEFPGQAVANVIDENVKLCRRLIVIVVPESLGFGLLKNLSEEQIAVYNALIQDGMKVILIELEKIEDYTAMPESIQYIRQKHGVIRWHGDFTEQSQCVKTKFWKTVRYHMPPRRCRPSPPVQLPQHTPCYRTTGERVGGHKVRHALMEGLSLRGGSQLEEDTFHRGRPL

SEQ ID NO: 79 - protein, 555 aa, 人工序列(Artificial Sequence)
  CynoIL36R-ECD mFc
DGCNDIFMKNEMLSASQPFAFNCTFPPITSGEVSVTWYKNSSKIPVSKIIQSRIHQDETWILFLPMEWGDSGVYQCVIKGRDSCHRIHVNLTVFEKQWCDTSVKGLPNLSDEYKQILHLGKDDSLTCHLHFPKSCILGPIKWYKDCNEITGERFTVLETRLLVSNVSAEDRGNYACQVILTHSGKQYEVLNGITVSITERAGYGGSVPKIIYPKNNSIEVQLGTTLIVDCNITDTKDNTNLRCWRVNNTLVDDYYNESKRIREGVETHASFREYNLYTVNITFLEVKMEDYGLPFMCHAGVSAAYIMLQLPAPDFRIEGRMDEPRGPTIKPCPPCKCPAPNLLGGPSVFIFPPKIKDVLMISLSPIVTCVVVDVSEDDPDVQISWFVNNVEVHTAQTQTHREDYNSTLRVVSALPIQHQDWMSGKEFKCKVNNKDLPAPIERTISKPKGSVRAPQVYVLPPPEEEMTKKQVTLTCMVTDFMPEDIYVEWTNNGKTELNYKNTEPVLDSDGSYFMYSKLRVEKKNWVERNSYSCSVVHEGLHNHHTTKSFSRTPGK

SEQ ID NO: 80 - protein, 553 aa, 人工序列(Artificial Sequence)
  CynoIL36R-ECD hFc
DGCNDIFMKNEMLSASQPFAFNCTFPPITSGEVSVTWYKNSSKIPVSKIIQSRIHQDETWILFLPMEWGDSGVYQCVIKGRDSCHRIHVNLTVFEKQWCDTSVKGLPNLSDEYKQILHLGKDDSLTCHLHFPKSCILGPIKWYKDCNEITGERFTVLETRLLVSNVSAEDRGNYACQVILTHSGKQYEVLNGITVSITERAGYGGSVPKIIYPKNNSIEVQLGTTLIVDCNITDTKDNTNLRCWRVNNTLVDDYYNESKRIREGVETHASFREYNLYTVNITFLEVKMEDYGLPFMCHAGVSAAYIMLQLPAPDFRIEGRMDPKSCDKTHTCPPCPAPELLGGPSVFLFPPKPKDTLMISRTPEVTCVVVDVSHEDPEVKFNWYVDGVEVHNAKTKPREEQYNSTYRVVSVLTVLHQDWLNGKEYKCKVSNKALPAPIEKTISKAKGQPREPQVYTLPPSRDELTKNQVSLTCLVKGFYPSDIAVEWESNGQPENNYKTTPPVLDSDGSFFLYSKLTVDKSRWQQGNVFSCSVMHEALHNHYTQKSLSLSPGK

SEQ ID NO: 81 - protein, 449 aa, 人工序列(Artificial Sequence)
  BI655130的重链
QVQLVQSGAEVKKPGASVKVSCKASGYSFTSSWIHWVKQAPGQGLEWMGEINPGNVRTNYNENFRNKVTMTVDTSISTAYMELSRLRSDDTAVYYCTVVFYGEPYFPYWGQGTLVTVSSASTKGPSVFPLAPSSKSTSGGTAALGCLVKDYFPEPVTVSWNSGALTSGVHTFPAVLQSSGLYSLSSVVTVPSSSLGTQTYICNVNHKPSNTKVDKRVEPKSCDKTHTCPPCPAPEAAGGPSVFLFPPKPKDTLMISRTPEVTCVVVDVSHEDPEVKFNWYVDGVEVHNAKTKPREEQYNSTYRVVSVLTVLHQDWLNGKEYKCKVSNKALPAPIEKTISKAKGQPREPQVYTLPPSREEMTKNQVSLTCLVKGFYPSDIAVEWESNGQPENNYKTTPPVLDSDGSFFLYSKLTVDKSRWQQGNVFSCSVMHEALHNHYTQKSLSLSPGK

SEQ ID NO: 82 - DNA, 1347 bp, 人工序列(Artificial Sequence)
  BI655130的重链
caggtgcagctggtgcagtctggcgccgaggtgaagaagccaggcgctagcgtgaaggtgtcttgcaaggccagcggctactctttcacctccagctggatccactgggtgaagcaggctccaggacagggactggagtggatgggcgagatcaatcctggcaacgtgagaacaaactacaatgagaactttcgcaataaggtgaccatgacagtggacaccagcatctctacagcctatatggagctgtccaggctgcggagcgacgataccgccgtgtactattgcacagtggtgttctacggcgagccatactttccctattggggccagggcaccctggtgacagtgtcttccgcctctaccaagggcccctccgtgttccctctggctccaagctctaagtccaccagcggaggaacagccgctctgggctgtctggtgaaggattatttcccagagcccgtgaccgtgtcctggaatagcggcgccctgacctccggagtgcatacatttcccgctgtgctgcagtccagcggcctgtacagcctgtcttccgtggtgaccgtgcctagctcttccctgggcacccagacatatatctgcaatgtgaaccacaagccttccaacacaaaggtggacaagagggtggagccaaagagctgtgataagacccatacatgccccccttgtcctgctccagaggctgctggaggaccatccgtgttcctgtttccacccaagcccaaggacaccctgatgatctctaggacccctgaggtgacatgcgtggtggtggacgtgtcccacgaggatccagaggtgaagtttaattggtacgtggatggcgtggaggtgcataacgctaagaccaagcctagggaggagcagtacaacagcacctatcgggtggtgtctgtgctgacagtgctgcaccaggactggctgaatggcaaggagtataagtgcaaggtgagcaacaaggccctgcccgctcctatcgagaagaccatctctaaggccaagggccagcccagagagcctcaggtgtacacactgcctccaagccgcgaggagatgaccaagaatcaggtgtctctgacatgtctggtgaagggcttctatccatctgacatcgctgtggagtgggagtccaacggccagcccgagaacaattacaagaccacaccccctgtgctggactctgatggctccttctttctgtattccaagctgaccgtggataagagccggtggcagcagggcaacgtgttctcctgttccgtgatgcatgaggccctgcacaaccattacacacagaagagcctgtctctgtccccaggcaag

SEQ ID NO: 83 - protein, 215 aa, 人工序列(Artificial Sequence)
  BI655130的轻链
QIVLTQSPGTLSLSPGERATMTCTASSSVSSSYFHWYQQKPGQAPRLWIYRTSRLASGVPDRFSGSGSGTDFTLTISRLEPEDAATYYCHQFHRSPLTFGAGTKLEIKRTVAAPSVFIFPPSDEQLKSGTASVVCLLNNFYPREAKVQWKVDNALQSGNSQESVTEQDSKDSTYSLSSTLTLSKADYEKHKVYACEVTHQGLSSPVTKSFNRGEC

SEQ ID NO: 84 - DNA, 645 bp, 人工序列(Artificial Sequence)
  BI655130的轻链
cagatcgtgctgacacagagccctggcaccctgagcctgtctccaggagagagggccaccatgacatgcaccgcttccagctccgtgtccagctcttacttccactggtatcagcagaagccaggacaggctccaaggctgtggatctacaggacctccaggctggctagcggagtgcctgaccggttctccggaagcggatctggcacagacttcaccctgaccatctccagactggagcccgaggacgccgctacctactattgccaccagttccatagaagccctctgacatttggcgccggcaccaagctggagatcaagcgcacagtggccgctccaagcgtgttcatctttcccccttctgacgagcagctgaagtctggcaccgcttccgtggtgtgcctgctgaacaatttctacccccgcgaggccaaggtgcagtggaaggtggataacgctctgcagtccggcaatagccaggagtctgtgacagagcaggactccaaggatagcacctattctctgtccagcacactgaccctgtctaaggccgattacgagaagcacaaggtgtatgcttgcgaggtgacacatcagggcctgtcttccccagtgaccaagtcctttaacaggggcgagtgt

SEQ ID NO: 85 - protein, 5 aa, 人工序列(Artificial Sequence)
  Kabat定义的小鼠、嵌合和人源化72C1抗体的VH-CDR1
SGYWN

SEQ ID NO: 86 - protein, 5 aa, 人工序列(Artificial Sequence)
  Kabat定义的小鼠、嵌合和人源化84C4抗体的VH-CDR1
SYWMN

SEQ ID NO: 87 - protein, 11 aa, 人工序列(Artificial Sequence)
  Kabat定义的小鼠、嵌合和人源化84C4抗体的VL-CDR1
RASQDIGNALN

SEQ ID NO: 88 - protein, 5 aa, 人工序列(Artificial Sequence)
  Kabat定义的小鼠和嵌合74B4D6抗体的VH-CDR1
NYWIH

SEQ ID NO: 89 - protein, 5 aa, 人工序列(Artificial Sequence)
  Kabat定义的小鼠和嵌合58A8D1抗体的VH-CDR1
SSWMH

SEQ ID NO: 90 - protein, 5 aa, 人工序列(Artificial Sequence)
  Kabat定义的小鼠和嵌合6G10抗体的VH-CDR1
RFAMS